European Patent Application EP 4 741 508 A2, published May 13, 2026. Title: Hyperactive Transposons and Transposases. Applicant: Probiogen AG. Application WO PCT/EP2020/070320, filed July 17, 2020. The sequence listing filed with the application follows.

SEQUENCE LISTING (28 sequences)

SEQ ID NO: 1 - DNA, 17 bp, Trichoplusia ni
  source 1..17: mol_type = other DNA
tgagtcaaaatgacgca

SEQ ID NO: 2 - DNA, 13 bp, Xenopus tropicalis
  source 1..13: mol_type = other DNA
tggcagtaaaagg

SEQ ID NO: 3 - DNA, 17 bp, Bombyx mori
  source 1..17: mol_type = other DNA
gggtatgttataccctg

SEQ ID NO: 4 - DNA, 16 bp, Myotis lucifugus
  source 1..16: mol_type = other DNA
gagccgtcttaactcg

SEQ ID NO: 5 - DNA, 16 bp, Myotis lucifugus
  source 1..16: mol_type = other DNA
cgagtgttctcgtttt

SEQ ID NO: 6 - DNA, 248 bp, Trichoplusia ni
  source 1..248: mol_type = other DNA
ccctagaaagatagtctgcgtaaaattgacgcatggctagctgaaatattgctctctctttctaaatagcgcgaatccgtcgctgtgcatttaggacatctcagtcgccgcttggagctcccgtgaggcgtgcttgtcaatgcggtaagtgtcactgattttgaactataacgaccgcgtgagtcaaaatgacgcatgattatcttttacgtgacttttaagatttaactcatacgataattgctagc

SEQ ID NO: 7 - DNA, 97 bp, Xenopus tropicalis
  source 1..97: mol_type = other DNA
cccttgatgtcaataccaaaccaaaagcagcgctaaggttgatccttaacctttttactgccaatgacgcatgggatacgtcgtggcagtaaaaggg

SEQ ID NO: 8 - DNA, 204 bp, Bombyx mori
  source 1..204: mol_type = other DNA
cccggcgagcatgaggcagggtatctcataccctggtaaaattttaaagttgtgtattttataaaattttcgtctgacaacactagcgcgctcagtagctggaggcaggagcgtgcgggaggggatagtggcgtgatcgcagtgtggcacgggacaccggcgagatattcgtgtgcaaacctgtttcgggtatgttataccctg

SEQ ID NO: 9 - DNA, 74 bp, Myotis lucifugus
  source 1..74: mol_type = other DNA
cacttggattgcgggaaacgagttaagtcggctcgcgtgaattgcgcgtactccgcgggagccgtcttaactcg

SEQ ID NO: 10 - DNA, 78 bp, Myotis lucifugus
  source 1..78: mol_type = other DNA
cacattgcgtaccgctcacgagttttctcgtgtttcgcgcgccatctgttaaggaccgctcacgagtgttctcgtttt

SEQ ID NO: 11 - DNA, 35 bp, Trichoplusia ni
  source 1..35: mol_type = other DNA
ccctagaaagatagtctgcgtaaaattgacgcatg

SEQ ID NO: 12 - DNA, 67 bp, Trichoplusia ni
  source 1..67: mol_type = other DNA
ttaacatgcgtcaattttacgcatgattatctttaacgtacgtcacaatatgattatctttctaggg

SEQ ID NO: 13 - DNA, 357 bp, Trichoplusia ni
  source 1..357: mol_type = other DNA
ccctagaaagatagtctgcgtaaaattgacgcatggctagctgaaatattgctctctctttctaaatagcgcgaatccgtcgctgtgcatttaggacatctcagtcgccgcttggagctcccgtgaggcgtgcttgtcaatgcggtaagtgtcactgattttgaactataacgaccgcgtgagtcaaaatgacgcatgattatcttttacgtgacttttaagatttaactcatacgataattatattgttatttcatgttctacttacgtgataacttattatatatatattttcttgttatagatatcgtgactaatatataataaactttgatgagaatcaatcttttctttcag

SEQ ID NO: 14 - DNA, 354 bp, Trichoplusia ni
  source 1..354: mol_type = other DNA
ttttctccttacgcatctgtgcggtatttcacaccgcatgggcagaatacaatggaaagtccctattgactcaggcctgtttaaaagttttgttactttatagaagaaattttgagtttttgtttttttttaataaataaataaacataaataaattgtttgttgaatttattattagtatgtaagtgtaaatataataaaacttaatatctattcaaattaataaataaacctcgatatacagaccgataaaacacggtggccacgcgttgggcctcggtggccacgcgtcatgcgtcaattttacgcatgattatctttaacgtacgtcacaatatgattatctttctaggg

SEQ ID NO: 15 - DNA, 248 bp, synthetic construct
  misc_feature 1..248: note = Transposon end
  source 1..248: mol_type = other DNA
ccctagaaagatagtctgcgtaaaattgacgcatggctagctgaaatattgctctctctttctaaatagcgcgaatccgtcgctgtgcatttaggacatctcagtcgccgcttggagctcccgtgaggcgtgcttgtcaatgcggtaagtgtcactgattttgaactataacgaccgcgtgcgtcaattttacgcatgattatcttttacgtgacttttaagatttaactcatacgataattgctagc

SEQ ID NO: 16 - DNA, 357 bp, synthetic construct
  misc_feature 1..357: note = Transposon end
  source 1..357: mol_type = other DNA
ccctagaaagatagtctgcgtaaaattgacgcatggctagctgaaatattgctctctctttctaaatagcgcgaatccgtcgctgtgcatttaggacatctcagtcgccgcttggagctcccgtgaggcgtgcttgtcaatgcggtaagtgtcactgattttgaactataacgaccgcgtgcgtcaattttacgcatgattatcttttacgtgacttttaagatttaactcatacgataattatattgttatttcatgttctacttacgtgataacttattatatatatattttcttgttatagatatcgtgactaatatataataaactttgatgagaatcaatcttttctttcag

SEQ ID NO: 17 - DNA, 1785 bp, Trichoplusia ni
  source 1..1785: mol_type = other DNA
  CDS 1..1782
atgggctctagcctggacgacgagcacattctgtctgccctgctgcagtccgacgatgaactcgtgggcgaagattccgactccgagatctctgaccacgtgtccgaggacgacgtgcagtctgataccgaggaagccttcatcgacgaggtgcacgaagtgcagcctacctcttccggctctgagatcctggacgagcagaacgtgatcgagcagcctggatcctctctggcctccaacagaatcctgacactgccccagagaaccatccggggcaagaacaagcactgctggtccacctccaagtctacccggcggtctagagtgtccgctctgaatattgtgcggtcccagaggggccccaccagaatgtgccggaacatctacgaccctctgctgtgtttcaagctgttcttcaccgacgagatcatcagcgagatcgtgaagtggaccaacgccgagatcagcctgaagcggcgggaatctatgaccggcgccaccttcagagacaccaacgaggatgagatctacgccttcttcggcatcctggtcatgacagccgtgcggaaggacaaccacatgtccaccgacgacctgttcgacagatccctgtccatggtgtacgtgtccgtgatgagccgggacagattcgacttcctgatccggtgcctgcggatggacgacaagtccatcagacccacactgcgcgagaacgacgtgttcacacctgtgcggaagatctgggacctgttcatccaccagtgcatccagaactacacccctggcgctcacctgaccatcgatgaacagctgctgggcttcagaggcagatgccccttcagaatgtacatccccaacaagccctctaagtacggcatcaagatcctgatgatgtgcgactccggcaccaagtacatgatcaacggcatgccctacctcggcagaggcacccaaacaaatggcgtgccactgggcgagtactatgtgaaagaactgtccaagcctgtgcacggctcctgcagaaacatcacctgtgacaactggttcaccagcattcctctggccaagaacctgctgcaagagccctacaagctgacaatcgtgggcaccgtgcggtccaacaagcgggaaattcctgaggtgctgaagaactctcggtccagacctgtgggcacctccatgttctgtttcgacggccctctgacactggtgtcctacaagcctaagcctgccaagatggtgtacctgctgtcctcctgtgacgaggacgccagcatcaatgagtccaccggcaagccccagatggtcatgtactacaaccagaccaaaggcggcgtggacaccctggaccagatgtgctctgtgatgacctgctccagaaagaccaacagatggcccatggctctgctgtacggcatgatcaatatcgcctgcatcaacagcttcatcatctactcccacaacgtgtcctccaagggcgagaaggtgcagtcccggaagaaattcatgcggaacctgtatatgtccctgacctccagcttcatgagaaagcggctggaagcccctactctgaagagatacctgcgggacaacatctccaacatcctgcctaacgaggtgcccggcaccagcgacgattctacagaggaacctgtgatgaagaagcggacctactgcacctactgtccctccaagatccggcggaaggccaacgcctcttgcaaaaagtgcaagaaagtgatctgccgcgagcacaacatcgacatgtgccagtcttgtttctga

SEQ ID NO: 18 - protein, 594 aa, Trichoplusia ni
MGSSLDDEHILSALLQSDDELVGEDSDSEISDHVSEDDVQSDTEEAFIDEVHEVQPTSSGSEILDEQNVIEQPGSSLASNRILTLPQRTIRGKNKHCWSTSKSTRRSRVSALNIVRSQRGPTRMCRNIYDPLLCFKLFFTDEIISEIVKWTNAEISLKRRESMTGATFRDTNEDEIYAFFGILVMTAVRKDNHMSTDDLFDRSLSMVYVSVMSRDRFDFLIRCLRMDDKSIRPTLRENDVFTPVRKIWDLFIHQCIQNYTPGAHLTIDEQLLGFRGRCPFRMYIPNKPSKYGIKILMMCDSGTKYMINGMPYLGRGTQTNGVPLGEYYVKELSKPVHGSCRNITCDNWFTSIPLAKNLLQEPYKLTIVGTVRSNKREIPEVLKNSRSRPVGTSMFCFDGPLTLVSYKPKPAKMVYLLSSCDEDASINESTGKPQMVMYYNQTKGGVDTLDQMCSVMTCSRKTNRWPMALLYGMINIACINSFIIYSHNVSSKGEKVQSRKKFMRNLYMSLTSSFMRKRLEAPTLKRYLRDNISNILPNEVPGTSDDSTEEPVMKKRTYCTYCPSKIRRKANASCKKCKKVICREHNIDMCQSCF

SEQ ID NO: 19 - DNA, 1785 bp, synthetic construct
  misc_feature 1..1785: note = Hyperactive Transposase
  source 1..1785: mol_type = other DNA
  CDS 1..1782
atgggcagctctctggacgacgagcacatcctgtctgccctgctgcagtctgacgatgaactcgtgggcgaagattccgactccgaggcctctgaccatgtgtctgaggacgacgtgcagtccgataccgaggaagccttcatcgacgaggtgcacgaagtgcagcctacctcttccggctctgagatcctggacgagcagaacgtgatcgagcagcctggatcctctctggcctccaacagaatcctgacactgccccagagaaccatccggggcaagaacaagcactgctggtccacctccaagtctacccggcggtctagagtgtccgctctgaatattgtgcggtccccgaggggccccaccagaatgtgccggaacatctacgaccctctgctgtgcttcaagctgttcttcaccgacgagatcatctccgagatcgtgaagtggaccaacgccgagatctctctgaagcggcgcgagtctatgaccggcgccaccttcagagacaccaacgaggatgagatctacgccttcttcggcatcctggtcgtcacagccgtgcggaaggacaaccacatgtccaccgacgacctgttcgacagatccctgtccatggtgtacgtgtccgtgatgagccgggacagattcgacttcctgatccggtgcctgcggatggacgacaagtccatcagacccacactgcgcgagaacgacgtgttcacacctgtgcggaagatctgggacctgttcatccaccagtgcatccagaactacacccctggcgctcacctgaccatcgacgaacagctgctgggcttcagaggcagatgccctttccggctgtacatccccaacaagccctctaagtacggcatcaagatcctgatgatgtgcgactccggcaccaagtacatgatcaacggcatgccctacctcggcagaggcacccaaacaaatggcgtgccactgggcgagtactacgtgaaagaactgtccaagcctgtgcacggctcctgcagaaacatcacctgtgacaactggttcaccagcattcctctggccaagaacctgctgcaagagccctacaagctgacaatcgtgggcaccgtgcggtccaacaagcgggaaattcctgaggtgctgaagaactctcggtccagacctgtgggcacctccatgttctgtttcgacggccctctgacactggtgtcctacaagcctaagcctgccaagatggtgtacctgctgtcctcctgtgacgaggacgccagcatcaatgagtccaccggcaagccccagatggtcatgtactacaaccagaccaaaggcggcgtggacaccctggaccagatgtgctctgtgatgacctgctccagaaagaccaaccggtggcctatggctctgctgtacggcatgatcaatatcgcctgcatcaacagcttcatcatctactcccacaacgtgtcctccaagggcgagaaggtgcagtcccggaagaaattcatgcggaacctgtatatgtccctgacctccagcttcatgagaaagcggctggaagcccctacactgaagagatacctgcgggacaacatctccaacatcctgcctagagaggtgcccggcaccagcgacgattctacagaggaacccgtgatgaagaagcggacctactgcacctactgtccctccaagatccggcggaaggccaacgcctcttgcaaaaagtgcaagaaagtgatctgccgcgagcacaacatcgacatgtgccagtcttgtttctga

SEQ ID NO: 20 - protein, 594 aa, synthetic construct
  REGION 1..594: note = Synthetic Construct
MGSSLDDEHILSALLQSDDELVGEDSDSEASDHVSEDDVQSDTEEAFIDEVHEVQPTSSGSEILDEQNVIEQPGSSLASNRILTLPQRTIRGKNKHCWSTSKSTRRSRVSALNIVRSPRGPTRMCRNIYDPLLCFKLFFTDEIISEIVKWTNAEISLKRRESMTGATFRDTNEDEIYAFFGILVVTAVRKDNHMSTDDLFDRSLSMVYVSVMSRDRFDFLIRCLRMDDKSIRPTLRENDVFTPVRKIWDLFIHQCIQNYTPGAHLTIDEQLLGFRGRCPFRLYIPNKPSKYGIKILMMCDSGTKYMINGMPYLGRGTQTNGVPLGEYYVKELSKPVHGSCRNITCDNWFTSIPLAKNLLQEPYKLTIVGTVRSNKREIPEVLKNSRSRPVGTSMFCFDGPLTLVSYKPKPAKMVYLLSSCDEDASINESTGKPQMVMYYNQTKGGVDTLDQMCSVMTCSRKTNRWPMALLYGMINIACINSFIIYSHNVSSKGEKVQSRKKFMRNLYMSLTSSFMRKRLEAPTLKRYLRDNISNILPREVPGTSDDSTEEPVMKKRTYCTYCPSKIRRKANASCKKCKKVICREHNIDMCQSCF

SEQ ID NO: 21 - DNA, 1785 bp, synthetic construct
  misc_feature 1..1785: note = hyperactive Transposase
  source 1..1785: mol_type = other DNA
  CDS 1..1782
atgggcagctctctggacgacgagcacatcctgtctgccctgctgcagtctgacgatgaactcgtgggcgaagattccgactccgaggcctctgaccatgtgtctgaggacgacgtgcagtccgataccgaggaagccttcatcgacgaggtgcacgaagtgcagcctacctcttccggctctgagatcctggacgagcagaacgtgatcgagcagcctggatcctctctggcctccaacagaatcctgacactgccccagagaaccatccggggcaagaacaagcactgctggtccacctccaagtctacccggcggtctagagtgtccgctctgaatattgtgcggtcccagaggggccccaccagaatgtgccggaacatctacgaccctctgctgtgcttcaagctgttcttcaccgacgagatcatctccgagatcgtgaagtggaccaacgccgagatctctctgaagcggcgcgagtctatgaccggcgccaccttcagagacaccaacgaggatgagatctacgccttcttcggcatcctggtcatgacagccgtgcggaaggacaaccacatgtccaccgacgacctgttcgacagatccctgtccatggtgtacgtgtccgtgatgagccgggacagattcgacttcctgatccggtgcctgcggatggacgacaagtccatcagacccacactgcgcgagaacgacgtgttcacacctgtgcggaagatctgggacctgttcatccaccagtgcatccagaactacacccctggcgctcacctgaccatcgacgaacagctgctgggcttcagaggcagatgccctttccggctgtacatccccaacaagccctctaagtacggcatcaagatcctgatgatgtgcgactccggcaccaagtacatgatcaacggcatgccctacctcggcagaggcacccaaacaaatggcgtgccactgggcgagtactacgtgaaagaactgtccaagcctgtgcacggctcctgcagaaacatcacctgtgacaactggttcaccagcattcctctggccaagaacctgctgcaagagccctacaagctgacaatcgtgggcaccgtgcggtccaacaagcgggaaattcctgaggtgctgaagaactctcggtccagacctgtgggcacctccatgttctgtttcgacggccctctgacactggtgtcctacaagcctaagcctgccaagatggtgtacctgctgtcctcctgtgacgaggacgccagcatcaatgagtccaccggcaagccccagatggtcatgtactacaaccagaccaaaggcggcgtggacaccctggaccagatgtgctctgtgatgacctgctccagaaagaccaaccggtggcctatggctctgctgtacggcatgatcaatatcgcctgcatcaacagcttcatcatctactcccacaacgtgtcctccaagggcgagaaggtgcagtcccggaagaaattcatgcggaacctgtatatgtccctgacctccagcttcatgagaaagcggctggaagcccctacactgaagagatacctgcgggacaacatctccaacatcctgcctagagaggtgcccggcaccagcgacgattctacagaggaacccgtgatgaagaagcggacctactgcacctactgtccctccaagatccggcggaaggccaacgcctcttgcaaaaagtgcaagaaagtgatctgccgcgagcacaacatcgacatgtgccagtcttgtttctga

SEQ ID NO: 22 - protein, 594 aa, synthetic construct
  REGION 1..594: note = Synthetic Construct
MGSSLDDEHILSALLQSDDELVGEDSDSEASDHVSEDDVQSDTEEAFIDEVHEVQPTSSGSEILDEQNVIEQPGSSLASNRILTLPQRTIRGKNKHCWSTSKSTRRSRVSALNIVRSQRGPTRMCRNIYDPLLCFKLFFTDEIISEIVKWTNAEISLKRRESMTGATFRDTNEDEIYAFFGILVMTAVRKDNHMSTDDLFDRSLSMVYVSVMSRDRFDFLIRCLRMDDKSIRPTLRENDVFTPVRKIWDLFIHQCIQNYTPGAHLTIDEQLLGFRGRCPFRLYIPNKPSKYGIKILMMCDSGTKYMINGMPYLGRGTQTNGVPLGEYYVKELSKPVHGSCRNITCDNWFTSIPLAKNLLQEPYKLTIVGTVRSNKREIPEVLKNSRSRPVGTSMFCFDGPLTLVSYKPKPAKMVYLLSSCDEDASINESTGKPQMVMYYNQTKGGVDTLDQMCSVMTCSRKTNRWPMALLYGMINIACINSFIIYSHNVSSKGEKVQSRKKFMRNLYMSLTSSFMRKRLEAPTLKRYLRDNISNILPREVPGTSDDSTEEPVMKKRTYCTYCPSKIRRKANASCKKCKKVICREHNIDMCQSCF

SEQ ID NO: 23 - DNA, 17 bp, Trichoplusia ni
  source 1..17: mol_type = other DNA
tgcgtaaaattgacgca

SEQ ID NO: 24 - DNA, 13 bp, Xenopus tropicalis
  source 1..13: mol_type = other DNA
cctttttactgcc

SEQ ID NO: 25 - DNA, 17 bp, Bombyx mori
  source 1..17: mol_type = other DNA
gggtatctcataccctg

SEQ ID NO: 26 - DNA, 16 bp, Mytois lucifugus
  source 1..16: mol_type = other DNA
cgagttaagtcggctc

SEQ ID NO: 27 - DNA, 16 bp, Mytois lucifugus
  source 1..16: mol_type = other DNA
cgagttttctcgtgtt

SEQ ID NO: 28 - DNA, 17 bp, synthetic construct
  misc_feature 1..17: note = piggyBac Transposon, Trichoplusia ni, artificial left internal repeat
  source 1..17: mol_type = other DNA
tgcgtcaattttacgca